European Patent Application EP 4 506 367 A1, published February 12, 2025. Title: AAV vector encoding anti-VEGF-A and ANG-2 bispecific antibody. Applicant: Starrygene Therapeutics Co., Ltd. The sequence listing filed with the application follows.

SEQUENCE LISTING (62 sequences)

SEQ ID NO: 1 - protein, 5 aa, synthetic construct
  REGION 1..5: note = VH VEGF-A G6-23 -CDR1
DYWIH

SEQ ID NO: 2 - protein, 17 aa, synthetic construct
  REGION 1..17: note = VH VEGF-A G6-23 -CDR2
GITPAGGYTYYADSVKG

SEQ ID NO: 3 - protein, 11 aa, synthetic construct
  REGION 1..11: note = VH VEGF-A G6-23 -CDR3
FVFFLPYAMDY

SEQ ID NO: 4 - protein, 11 aa, synthetic construct
  REGION 1..11: note = VL VEGF-A G6-23 -CDR1
RASQDVSTAVA

SEQ ID NO: 5 - protein, 7 aa, synthetic construct
  REGION 1..7: note = VL VEGF-A G6-23 -CDR2
SASFLYS

SEQ ID NO: 6 - protein, 9 aa, synthetic construct
  REGION 1..9: note = VL VEGF-A G6-23 -CDR3
KQGYANPWT

SEQ ID NO: 7 - protein, 5 aa, synthetic construct
  REGION 1..5: note = VH ANG-2 3.19.3 -CDR1
NYGMH

SEQ ID NO: 8 - protein, 17 aa, synthetic construct
  REGION 1..17: note = VH ANG-2 3.19.3 -CDR2
VISHDGNNKYYVDSVKG

SEQ ID NO: 9 - protein, 14 aa, synthetic construct
  REGION 1..14: note = VH ANG-2 3.19.3 -CDR3
EGIDFWSGLNWFDP

SEQ ID NO: 10 - protein, 12 aa, synthetic construct
  REGION 1..12: note = VL ANG-2 3.19.3 -CDR1
RASQSITGSYLA

SEQ ID NO: 11 - protein, 7 aa, synthetic construct
  REGION 1..7: note = VL ANG-2 3.19.3 -CDR2
GASSWAT

SEQ ID NO: 12 - protein, 9 aa, synthetic construct
  REGION 1..9: note = VL ANG-2 3.19.3 -CDR3
QQYSSSPIT

SEQ ID NO: 13 - protein, 120 aa, synthetic construct
  REGION 1..120: note = VH VEGF-A G6-23
EVQLVESGGGLVQPGGSLRLSCAASGFTISDYWIHWVRQAPGKGLEWVAGITPAGGYTYYADSVKGRFTISADTSKNTAYLQMNSLRAEDTAVYYCARFVFFLPYAMDYWGQGTLVTVSS

SEQ ID NO: 14 - protein, 108 aa, synthetic construct
  REGION 1..108: note = VL VEGF-A G6-23
DIQMTQSPSSLSASVGDRVTITCRASQDVSTAVAWYQQKPGKAPKLLIYSASFLYSGVPSRFSGSGSGTDFTLTISSLQPEDFATYYCKQGYANPWTFGQGTKVEIKR

SEQ ID NO: 15 - protein, 124 aa, synthetic construct
  REGION 1..124: note = VH ANG-2 3.19.3
QVQLVESGGGVVQPGRSLRLSCAASGFTFTNYGMHWGRQAPGKGLEWVAVISHDGNNKYYVDSVKGRFTISRDNSKNTLYLQMNSLRAEDTAVYYCAREGIDFWSGLNWFDPWGQGTLVTVSSA

SEQ ID NO: 16 - protein, 109 aa, synthetic construct
  REGION 1..109: note = VL ANG-2 3.19.3
EIVLTQSPGTLSLSPGERATLSCRASQSITGSYLAWYQQKPGQAPRLLICGASSWATGIPDRFSGSGSGTDFTLTISRLEPEDFAVYYCQQYSSSPITFGQGTRLEIKR

SEQ ID NO: 17 - protein, 496 aa, synthetic construct
  REGION 1..496: note = VH VEGF-A- (G4S)3-VL VEGF-A- G4S-VH ANG-2- (G4S)3-VL ANG-2
EVQLVESGGGLVQPGGSLRLSCAASGFTISDYWIHWVRQAPGKGLEWVAGITPAGGYTYYADSVKGRFTISADTSKNTAYLQMNSLRAEDTAVYYCARFVFFLPYAMDYWGQGTLVTVSSGGGGSGGGGSGGGGSDIQMTQSPSSLSASVGDRVTITCRASQDVSTAVAWYQQKPGKAPKLLIYSASFLYSGVPSRFSGSGSGTDFTLTISSLQPEDFATYYCKQGYANPWTFGQGTKVEIKRGGGGSQVQLVESGGGVVQPGRSLRLSCAASGFTFTNYGMHWGRQAPGKGLEWVAVISHDGNNKYYVDSVKGRFTISRDNSKNTLYLQMNSLRAEDTAVYYCAREGIDFWSGLNWFDPWGQGTLVTVSSAGGGGSGGGGSGGGGSEIVLTQSPGTLSLSPGERATLSCRASQSITGSYLAWYQQKPGQAPRLLICGASSWATGIPDRFSGSGSGTDFTLTISRLEPEDFAVYYCQQYSSSPITFGQGTRLEIKR

SEQ ID NO: 18 - protein, 486 aa, synthetic construct
  REGION 1..486: note = VL ANG-2-G4S-VH VEGF-A-(G4S)3-VL VEGF-A-G4S-VH ANG-2
EIVLTQSPGTLSLSPGERATLSCRASQSITGSYLAWYQQKPGQAPRLLICGASSWATGIPDRFSGSGSGTDFTLTISRLEPEDFAVYYCQQYSSSPITFGQGTRLEIKRGGGGSEVQLVESGGGLVQPGGSLRLSCAASGFTISDYWIHWVRQAPGKGLEWVAGITPAGGYTYYADSVKGRFTISADTSKNTAYLQMNSLRAEDTAVYYCARFVFFLPYAMDYWGQGTLVTVSSGGGGSGGGGSGGGGSDIQMTQSPSSLSASVGDRVTITCRASQDVSTAVAWYQQKPGKAPKLLIYSASFLYSGVPSRFSGSGSGTDFTLTISSLQPEDFATYYCKQGYANPWTFGQGTKVEIKRGGGGSQVQLVESGGGVVQPGRSLRLSCAASGFTFTNYGMHWGRQAPGKGLEWVAVISHDGNNKYYVDSVKGRFTISRDNSKNTLYLQMNSLRAEDTAVYYCAREGIDFWSGLNWFDPWGQGTLVTVSSA

SEQ ID NO: 19 - protein, 486 aa, synthetic construct
  REGION 1..486: note = VL VEGF-A-G4S -VH ANG-2-(G4S)3-VL ANG-2-G4S -VH VEGF-A
DIQMTQSPSSLSASVGDRVTITCRASQDVSTAVAWYQQKPGKAPKLLIYSASFLYSGVPSRFSGSGSGTDFTLTISSLQPEDFATYYCKQGYANPWTFGQGTKVEIKRGGGGSQVQLVESGGGVVQPGRSLRLSCAASGFTFTNYGMHWGRQAPGKGLEWVAVISHDGNNKYYVDSVKGRFTISRDNSKNTLYLQMNSLRAEDTAVYYCAREGIDFWSGLNWFDPWGQGTLVTVSSAGGGGSGGGGSGGGGSEIVLTQSPGTLSLSPGERATLSCRASQSITGSYLAWYQQKPGQAPRLLICGASSWATGIPDRFSGSGSGTDFTLTISRLEPEDFAVYYCQQYSSSPITFGQGTRLEIKRGGGGSEVQLVESGGGLVQPGGSLRLSCAASGFTISDYWIHWVRQAPGKGLEWVAGITPAGGYTYYADSVKGRFTISADTSKNTAYLQMNSLRAEDTAVYYCARFVFFLPYAMDYWGQGTLVTVSS

SEQ ID NO: 20 - protein, 520 aa, synthetic construct
  REGION 1..520: note = CD5-sp-VH VEGF-A- (G4S)3-VL VEGF-A- G4S-VH ANG-2- (G4S)3-VL ANG-2
MPMGSLQPLATLYLLGMLVASCLGEVQLVESGGGLVQPGGSLRLSCAASGFTISDYWIHWVRQAPGKGLEWVAGITPAGGYTYYADSVKGRFTISADTSKNTAYLQMNSLRAEDTAVYYCARFVFFLPYAMDYWGQGTLVTVSSGGGGSGGGGSGGGGSDIQMTQSPSSLSASVGDRVTITCRASQDVSTAVAWYQQKPGKAPKLLIYSASFLYSGVPSRFSGSGSGTDFTLTISSLQPEDFATYYCKQGYANPWTFGQGTKVEIKRGGGGSQVQLVESGGGVVQPGRSLRLSCAASGFTFTNYGMHWGRQAPGKGLEWVAVISHDGNNKYYVDSVKGRFTISRDNSKNTLYLQMNSLRAEDTAVYYCAREGIDFWSGLNWFDPWGQGTLVTVSSAGGGGSGGGGSGGGGSEIVLTQSPGTLSLSPGERATLSCRASQSITGSYLAWYQQKPGQAPRLLICGASSWATGIPDRFSGSGSGTDFTLTISRLEPEDFAVYYCQQYSSSPITFGQGTRLEIKR

SEQ ID NO: 21 - protein, 510 aa, synthetic construct
  REGION 1..510: note = CD5-sp-VL ANG-2-G4S-VH VEGF-A-(G4S)3-VL VEGF-A-G4S-VH ANG-2
MPMGSLQPLATLYLLGMLVASCLGEIVLTQSPGTLSLSPGERATLSCRASQSITGSYLAWYQQKPGQAPRLLICGASSWATGIPDRFSGSGSGTDFTLTISRLEPEDFAVYYCQQYSSSPITFGQGTRLEIKRGGGGSEVQLVESGGGLVQPGGSLRLSCAASGFTISDYWIHWVRQAPGKGLEWVAGITPAGGYTYYADSVKGRFTISADTSKNTAYLQMNSLRAEDTAVYYCARFVFFLPYAMDYWGQGTLVTVSSGGGGSGGGGSGGGGSDIQMTQSPSSLSASVGDRVTITCRASQDVSTAVAWYQQKPGKAPKLLIYSASFLYSGVPSRFSGSGSGTDFTLTISSLQPEDFATYYCKQGYANPWTFGQGTKVEIKRGGGGSQVQLVESGGGVVQPGRSLRLSCAASGFTFTNYGMHWGRQAPGKGLEWVAVISHDGNNKYYVDSVKGRFTISRDNSKNTLYLQMNSLRAEDTAVYYCAREGIDFWSGLNWFDPWGQGTLVTVSSA

SEQ ID NO: 22 - protein, 510 aa, synthetic construct
  REGION 1..510: note = CD5-sp-VL VEGF-A-G4S -VH ANG-2-(G4S)3-VL ANG-2-G4S -VH VEGF-A
MPMGSLQPLATLYLLGMLVASCLGDIQMTQSPSSLSASVGDRVTITCRASQDVSTAVAWYQQKPGKAPKLLIYSASFLYSGVPSRFSGSGSGTDFTLTISSLQPEDFATYYCKQGYANPWTFGQGTKVEIKRGGGGSQVQLVESGGGVVQPGRSLRLSCAASGFTFTNYGMHWGRQAPGKGLEWVAVISHDGNNKYYVDSVKGRFTISRDNSKNTLYLQMNSLRAEDTAVYYCAREGIDFWSGLNWFDPWGQGTLVTVSSAGGGGSGGGGSGGGGSEIVLTQSPGTLSLSPGERATLSCRASQSITGSYLAWYQQKPGQAPRLLICGASSWATGIPDRFSGSGSGTDFTLTISRLEPEDFAVYYCQQYSSSPITFGQGTRLEIKRGGGGSEVQLVESGGGLVQPGGSLRLSCAASGFTISDYWIHWVRQAPGKGLEWVAGITPAGGYTYYADSVKGRFTISADTSKNTAYLQMNSLRAEDTAVYYCARFVFFLPYAMDYWGQGTLVTVSS

SEQ ID NO: 23 - protein, 24 aa, synthetic construct
  REGION 1..24: note = CD5-sp
MPMGSLQPLATLYLLGMLVASCLG

SEQ ID NO: 24 - DNA, 15 bp, synthetic construct
  misc_feature 1..15: note = VH VEGF-A G6-23 -CDR1
  source 1..15: mol_type = other DNA
gactactggattcac

SEQ ID NO: 25 - DNA, 51 bp, synthetic construct
  misc_feature 1..51: note = VH VEGF-A G6-23 -CDR2
  source 1..51: mol_type = other DNA
ggaatcaccccagcaggaggctacacatactatgccgacagcgtgaagggc

SEQ ID NO: 26 - DNA, 33 bp, synthetic construct
  misc_feature 1..33: note = VH VEGF-A G6-23 -CDR3
  source 1..33: mol_type = other DNA
ttcgtgttcttcctgccatacgccatggattat

SEQ ID NO: 27 - DNA, 360 bp, synthetic construct
  misc_feature 1..360: note = VH VEGF-A G6-23
  source 1..360: mol_type = other DNA
gaggtgcagctggtggagagcggaggaggactggtgcagccaggaggctccctgcggctgtcttgcgccgccagcggctttaccatctccgactactggattcactgggtgagacaggcacctggcaagggactggagtgggtggcaggaatcaccccagcaggaggctacacatactatgccgacagcgtgaagggccggttcaccatctccgccgatacctctaagaacacagcctatctgcagatgaactccctgcgggccgaggacacagccgtgtactattgcgccagattcgtgttcttcctgccatacgccatggattattggggccagggcaccctggtgacagtgagctcc

SEQ ID NO: 28 - DNA, 33 bp, synthetic construct
  misc_feature 1..33: note = VL VEGF-A G6-23 -CDR1
  source 1..33: mol_type = other DNA
agagcaagccaggacgtgagcaccgcagtggca

SEQ ID NO: 29 - DNA, 21 bp, synthetic construct
  misc_feature 1..21: note = VL VEGF-A G6-23 -CDR2
  source 1..21: mol_type = other DNA
tccgcctctttcctgtattct

SEQ ID NO: 30 - DNA, 27 bp, synthetic construct
  misc_feature 1..27: note = VL VEGF-A G6-23 -CDR3
  source 1..27: mol_type = other DNA
aagcagggctatgccaatccatggacc

SEQ ID NO: 31 - DNA, 324 bp, synthetic construct
  misc_feature 1..324: note = VL VEGF-A G6-23
  source 1..324: mol_type = other DNA
gatattcagatgacacagtccccatctagcctgtctgccagcgtgggcgacagggtgaccatcacatgtagagcaagccaggacgtgagcaccgcagtggcatggtaccagcagaagcctggcaaggccccaaagctgctgatctactccgcctctttcctgtattctggcgtgccaagcaggtttagcgggtccggatctggaaccgacttcaccctgacaatctcctctctgcagcctgaggattttgccacatactattgcaagcagggctatgccaatccatggaccttcggccagggcacaaaggtggagatcaagagg

SEQ ID NO: 32 - DNA, 15 bp, synthetic construct
  misc_feature 1..15: note = VH ANG-2 3.19.3 -CDR1
  source 1..15: mol_type = other DNA
aactatggaatgcac

SEQ ID NO: 33 - DNA, 51 bp, synthetic construct
  misc_feature 1..51: note = VH ANG-2 3.19.3 -CDR2
  source 1..51: mol_type = other DNA
gtgatcagccacgacggcaacaacaagtactacgtggacagcgtgaagggc

SEQ ID NO: 34 - DNA, 42 bp, synthetic construct
  misc_feature 1..42: note = VH ANG-2 3.19.3 -CDR3
  source 1..42: mol_type = other DNA
gagggcatcgacttttggagcggcctgaattggttcgaccct

SEQ ID NO: 35 - DNA, 372 bp, synthetic construct
  misc_feature 1..372: note = VH ANG-2 3.19.3
  source 1..372: mol_type = other DNA
caggtgcagctggttgaatctggtggcggagttgtgcagcctggcagaagcctgagactgtcttgtgccgccagcggcttcaccttcaccaactatggaatgcactggggcagacaggcccctggcaaaggacttgaatgggtcgccgtgatcagccacgacggcaacaacaagtactacgtggacagcgtgaagggcagattcaccatcagccgggacaacagcaagaacaccctgtacctgcagatgaacagcctgagagccgaggacaccgccgtgtactattgtgccagagagggcatcgacttttggagcggcctgaattggttcgacccttggggacagggcaccctggttacagtttcttctgcc

SEQ ID NO: 36 - DNA, 36 bp, synthetic construct
  misc_feature 1..36: note = VL ANG-2 3.19.3 -CDR1
  source 1..36: mol_type = other DNA
agagccagccagagcatcaccggctcttacctggct

SEQ ID NO: 37 - DNA, 21 bp, synthetic construct
  misc_feature 1..21: note = VL ANG-2 3.19.3 -CDR2
  source 1..21: mol_type = other DNA
ggcgcctcttcttgggccacc

SEQ ID NO: 38 - DNA, 27 bp, synthetic construct
  misc_feature 1..27: note = VL ANG-2 3.19.3 -CDR3
  source 1..27: mol_type = other DNA
cagcagtacagcagcagccccatcacc

SEQ ID NO: 39 - DNA, 327 bp, synthetic construct
  misc_feature 1..327: note = VL ANG-2 3.19.3
  source 1..327: mol_type = other DNA
gagatcgtgctgacacagagccctggcacactgtcactgtctccaggcgaaagagccacactgagctgtagagccagccagagcatcaccggctcttacctggcttggtatcagcagaagcctggacaggcccctagactgctgatttgtggcgcctcttcttgggccaccggcattcccgatagattttctggcagcggctccggcaccgacttcaccctgacaatcagcagactggaacccgaggacttcgccgtgtactactgccagcagtacagcagcagccccatcacctttggccagggcacaagactggaaatcaagcgg

SEQ ID NO: 40 - DNA, 1488 bp, synthetic construct
  misc_feature 1..1488: note = VH VEGF-A- (G4S)3-VL VEGF-A- G4S-VH ANG-2- (G4S)3-VL ANG-2
  source 1..1488: mol_type = other DNA
gaggtgcagctggtggagagcggaggaggactggtgcagccaggaggctccctgcggctgtcttgcgccgccagcggctttaccatctccgactactggattcactgggtgagacaggcacctggcaagggactggagtgggtggcaggaatcaccccagcaggaggctacacatactatgccgacagcgtgaagggccggttcaccatctccgccgatacctctaagaacacagcctatctgcagatgaactccctgcgggccgaggacacagccgtgtactattgcgccagattcgtgttcttcctgccatacgccatggattattggggccagggcaccctggtgacagtgagctccggtggaggtggctccggtggcggtggcagcggcggtggcggctctgatattcagatgacacagtccccatctagcctgtctgccagcgtgggcgacagggtgaccatcacatgtagagcaagccaggacgtgagcaccgcagtggcatggtaccagcagaagcctggcaaggccccaaagctgctgatctactccgcctctttcctgtattctggcgtgccaagcaggtttagcgggtccggatctggaaccgacttcaccctgacaatctcctctctgcagcctgaggattttgccacatactattgcaagcagggctatgccaatccatggaccttcggccagggcacaaaggtggagatcaagaggggcggagggggctctcaggtgcagctggttgaatctggtggcggagttgtgcagcctggcagaagcctgagactgtcttgtgccgccagcggcttcaccttcaccaactatggaatgcactggggcagacaggcccctggcaaaggacttgaatgggtcgccgtgatcagccacgacggcaacaacaagtactacgtggacagcgtgaagggcagattcaccatcagccgggacaacagcaagaacaccctgtacctgcagatgaacagcctgagagccgaggacaccgccgtgtactattgtgccagagagggcatcgacttttggagcggcctgaattggttcgacccttggggacagggcaccctggttacagtttcttctgccggtggaggtggctccggtggcggtggcagcggcggtggcggctctgagatcgtgctgacacagagccctggcacactgtcactgtctccaggcgaaagagccacactgagctgtagagccagccagagcatcaccggctcttacctggcttggtatcagcagaagcctggacaggcccctagactgctgatttgtggcgcctcttcttgggccaccggcattcccgatagattttctggcagcggctccggcaccgacttcaccctgacaatcagcagactggaacccgaggacttcgccgtgtactactgccagcagtacagcagcagccccatcacctttggccagggcacaagactggaaatcaagcgg

SEQ ID NO: 41 - DNA, 1560 bp, synthetic construct
  misc_feature 1..1560: note = CD5-sp-VH VEGF-A- (G4S)3-VL VEGF-A- G4S-VH ANG-2- (G4S)3-VL ANG-2
  source 1..1560: mol_type = other DNA
atgccaatggggtccctacaacccctggcaacactatatctgctaggtatgctcgtggcctcctgtttaggagaggtgcagctggtggagagcggaggaggactggtgcagccaggaggctccctgcggctgtcttgcgccgccagcggctttaccatctccgactactggattcactgggtgagacaggcacctggcaagggactggagtgggtggcaggaatcaccccagcaggaggctacacatactatgccgacagcgtgaagggccggttcaccatctccgccgatacctctaagaacacagcctatctgcagatgaactccctgcgggccgaggacacagccgtgtactattgcgccagattcgtgttcttcctgccatacgccatggattattggggccagggcaccctggtgacagtgagctccggtggaggtggctccggtggcggtggcagcggcggtggcggctctgatattcagatgacacagtccccatctagcctgtctgccagcgtgggcgacagggtgaccatcacatgtagagcaagccaggacgtgagcaccgcagtggcatggtaccagcagaagcctggcaaggccccaaagctgctgatctactccgcctctttcctgtattctggcgtgccaagcaggtttagcgggtccggatctggaaccgacttcaccctgacaatctcctctctgcagcctgaggattttgccacatactattgcaagcagggctatgccaatccatggaccttcggccagggcacaaaggtggagatcaagaggggcggagggggctctcaggtgcagctggttgaatctggtggcggagttgtgcagcctggcagaagcctgagactgtcttgtgccgccagcggcttcaccttcaccaactatggaatgcactggggcagacaggcccctggcaaaggacttgaatgggtcgccgtgatcagccacgacggcaacaacaagtactacgtggacagcgtgaagggcagattcaccatcagccgggacaacagcaagaacaccctgtacctgcagatgaacagcctgagagccgaggacaccgccgtgtactattgtgccagagagggcatcgacttttggagcggcctgaattggttcgacccttggggacagggcaccctggttacagtttcttctgccggtggaggtggctccggtggcggtggcagcggcggtggcggctctgagatcgtgctgacacagagccctggcacactgtcactgtctccaggcgaaagagccacactgagctgtagagccagccagagcatcaccggctcttacctggcttggtatcagcagaagcctggacaggcccctagactgctgatttgtggcgcctcttcttgggccaccggcattcccgatagattttctggcagcggctccggcaccgacttcaccctgacaatcagcagactggaacccgaggacttcgccgtgtactactgccagcagtacagcagcagccccatcacctttggccagggcacaagactggaaatcaagcgg

SEQ ID NO: 42 - DNA, 72 bp, synthetic construct
  misc_feature 1..72: note = CD5-sp
  source 1..72: mol_type = other DNA
atgccaatggggtccctacaacccctggcaacactatatctgctaggtatgctcgtggcctcctgtttagga

SEQ ID NO: 43 - DNA, 1458 bp, synthetic construct
  misc_feature 1..1458: note = VL ANG-2-G4S-VH VEGF-A-(G4S)3-VL VEGF-A-G4S-VH ANG-2
  source 1..1458: mol_type = other DNA
gagatcgtgctgacacagagccctggcacactgtcactgtctccaggcgaaagagccacactgagctgtagagccagccagagcatcaccggctcttacctggcttggtatcagcagaagcctggacaggcccctagactgctgatttgtggcgcctcttcttgggccaccggcattcccgatagattttctggcagcggctccggcaccgacttcaccctgacaatcagcagactggaacccgaggacttcgccgtgtactactgccagcagtacagcagcagccccatcacctttggccagggcacaagactggaaatcaagcggggcggagggggctctgaggtgcagctggtggagagcggaggaggactggtgcagccaggaggctccctgcggctgtcttgcgccgccagcggctttaccatctccgactactggattcactgggtgagacaggcacctggcaagggactggagtgggtggcaggaatcaccccagcaggaggctacacatactatgccgacagcgtgaagggccggttcaccatctccgccgatacctctaagaacacagcctatctgcagatgaactccctgcgggccgaggacacagccgtgtactattgcgccagattcgtgttcttcctgccatacgccatggattattggggccagggcaccctggtgacagtgagctccggtggaggtggctccggtggcggtggcagcggcggtggcggctctgatattcagatgacacagtccccatctagcctgtctgccagcgtgggcgacagggtgaccatcacatgtagagcaagccaggacgtgagcaccgcagtggcatggtaccagcagaagcctggcaaggccccaaagctgctgatctactccgcctctttcctgtattctggcgtgccaagcaggtttagcgggtccggatctggaaccgacttcaccctgacaatctcctctctgcagcctgaggattttgccacatactattgcaagcagggctatgccaatccatggaccttcggccagggcacaaaggtggagatcaagaggggcggagggggctctcaggtgcagctggttgaatctggtggcggagttgtgcagcctggcagaagcctgagactgtcttgtgccgccagcggcttcaccttcaccaactatggaatgcactggggcagacaggcccctggcaaaggacttgaatgggtcgccgtgatcagccacgacggcaacaacaagtactacgtggacagcgtgaagggcagattcaccatcagccgggacaacagcaagaacaccctgtacctgcagatgaacagcctgagagccgaggacaccgccgtgtactattgtgccagagagggcatcgacttttggagcggcctgaattggttcgacccttggggacagggcaccctggttacagtttcttctgcc

SEQ ID NO: 44 - DNA, 1530 bp, synthetic construct
  misc_feature 1..1530: note = CD5-sp-VL ANG-2-G4S-VH VEGF-A-(G4S)3-VL VEGF-A-G4S-VH ANG-2
  source 1..1530: mol_type = other DNA
atgccaatggggtccctacaacccctggcaacactatatctgctaggtatgctcgtggcctcctgtttaggagagatcgtgctgacacagagccctggcacactgtcactgtctccaggcgaaagagccacactgagctgtagagccagccagagcatcaccggctcttacctggcttggtatcagcagaagcctggacaggcccctagactgctgatttgtggcgcctcttcttgggccaccggcattcccgatagattttctggcagcggctccggcaccgacttcaccctgacaatcagcagactggaacccgaggacttcgccgtgtactactgccagcagtacagcagcagccccatcacctttggccagggcacaagactggaaatcaagcggggcggagggggctctgaggtgcagctggtggagagcggaggaggactggtgcagccaggaggctccctgcggctgtcttgcgccgccagcggctttaccatctccgactactggattcactgggtgagacaggcacctggcaagggactggagtgggtggcaggaatcaccccagcaggaggctacacatactatgccgacagcgtgaagggccggttcaccatctccgccgatacctctaagaacacagcctatctgcagatgaactccctgcgggccgaggacacagccgtgtactattgcgccagattcgtgttcttcctgccatacgccatggattattggggccagggcaccctggtgacagtgagctccggtggaggtggctccggtggcggtggcagcggcggtggcggctctgatattcagatgacacagtccccatctagcctgtctgccagcgtgggcgacagggtgaccatcacatgtagagcaagccaggacgtgagcaccgcagtggcatggtaccagcagaagcctggcaaggccccaaagctgctgatctactccgcctctttcctgtattctggcgtgccaagcaggtttagcgggtccggatctggaaccgacttcaccctgacaatctcctctctgcagcctgaggattttgccacatactattgcaagcagggctatgccaatccatggaccttcggccagggcacaaaggtggagatcaagaggggcggagggggctctcaggtgcagctggttgaatctggtggcggagttgtgcagcctggcagaagcctgagactgtcttgtgccgccagcggcttcaccttcaccaactatggaatgcactggggcagacaggcccctggcaaaggacttgaatgggtcgccgtgatcagccacgacggcaacaacaagtactacgtggacagcgtgaagggcagattcaccatcagccgggacaacagcaagaacaccctgtacctgcagatgaacagcctgagagccgaggacaccgccgtgtactattgtgccagagagggcatcgacttttggagcggcctgaattggttcgacccttggggacagggcaccctggttacagtttcttctgcc

SEQ ID NO: 45 - DNA, 1458 bp, synthetic construct
  misc_feature 1..1458: note = VL VEGF-A-G4S -VH ANG-2-(G4S)3-VL ANG-2-G4S -VH VEGF-A
  source 1..1458: mol_type = other DNA
gatattcagatgacacagtccccatctagcctgtctgccagcgtgggcgacagggtgaccatcacatgtagagcaagccaggacgtgagcaccgcagtggcatggtaccagcagaagcctggcaaggccccaaagctgctgatctactccgcctctttcctgtattctggcgtgccaagcaggtttagcgggtccggatctggaaccgacttcaccctgacaatctcctctctgcagcctgaggattttgccacatactattgcaagcagggctatgccaatccatggaccttcggccagggcacaaaggtggagatcaagaggggcggagggggctctcaggtgcagctggttgaatctggtggcggagttgtgcagcctggcagaagcctgagactgtcttgtgccgccagcggcttcaccttcaccaactatggaatgcactggggcagacaggcccctggcaaaggacttgaatgggtcgccgtgatcagccacgacggcaacaacaagtactacgtggacagcgtgaagggcagattcaccatcagccgggacaacagcaagaacaccctgtacctgcagatgaacagcctgagagccgaggacaccgccgtgtactattgtgccagagagggcatcgacttttggagcggcctgaattggttcgacccttggggacagggcaccctggttacagtttcttctgccggtggaggtggctccggtggcggtggcagcggcggtggcggctctgagatcgtgctgacacagagccctggcacactgtcactgtctccaggcgaaagagccacactgagctgtagagccagccagagcatcaccggctcttacctggcttggtatcagcagaagcctggacaggcccctagactgctgatttgtggcgcctcttcttgggccaccggcattcccgatagattttctggcagcggctccggcaccgacttcaccctgacaatcagcagactggaacccgaggacttcgccgtgtactactgccagcagtacagcagcagccccatcacctttggccagggcacaagactggaaatcaagcggggcggagggggctctgaggtgcagctggtggagagcggaggaggactggtgcagccaggaggctccctgcggctgtcttgcgccgccagcggctttaccatctccgactactggattcactgggtgagacaggcacctggcaagggactggagtgggtggcaggaatcaccccagcaggaggctacacatactatgccgacagcgtgaagggccggttcaccatctccgccgatacctctaagaacacagcctatctgcagatgaactccctgcgggccgaggacacagccgtgtactattgcgccagattcgtgttcttcctgccatacgccatggattattggggccagggcaccctggtgacagtgagctcc

SEQ ID NO: 46 - DNA, 1530 bp, synthetic construct
  misc_feature 1..1530: note = CD5-sp-VL VEGF-A-G4S -VH ANG-2-(G4S)3-VL ANG-2-G4S -VH VEGF-A
  source 1..1530: mol_type = other DNA
atgccaatggggtccctacaacccctggcaacactatatctgctaggtatgctcgtggcctcctgtttaggagatattcagatgacacagtccccatctagcctgtctgccagcgtgggcgacagggtgaccatcacatgtagagcaagccaggacgtgagcaccgcagtggcatggtaccagcagaagcctggcaaggccccaaagctgctgatctactccgcctctttcctgtattctggcgtgccaagcaggtttagcgggtccggatctggaaccgacttcaccctgacaatctcctctctgcagcctgaggattttgccacatactattgcaagcagggctatgccaatccatggaccttcggccagggcacaaaggtggagatcaagaggggcggagggggctctcaggtgcagctggttgaatctggtggcggagttgtgcagcctggcagaagcctgagactgtcttgtgccgccagcggcttcaccttcaccaactatggaatgcactggggcagacaggcccctggcaaaggacttgaatgggtcgccgtgatcagccacgacggcaacaacaagtactacgtggacagcgtgaagggcagattcaccatcagccgggacaacagcaagaacaccctgtacctgcagatgaacagcctgagagccgaggacaccgccgtgtactattgtgccagagagggcatcgacttttggagcggcctgaattggttcgacccttggggacagggcaccctggttacagtttcttctgccggtggaggtggctccggtggcggtggcagcggcggtggcggctctgagatcgtgctgacacagagccctggcacactgtcactgtctccaggcgaaagagccacactgagctgtagagccagccagagcatcaccggctcttacctggcttggtatcagcagaagcctggacaggcccctagactgctgatttgtggcgcctcttcttgggccaccggcattcccgatagattttctggcagcggctccggcaccgacttcaccctgacaatcagcagactggaacccgaggacttcgccgtgtactactgccagcagtacagcagcagccccatcacctttggccagggcacaagactggaaatcaagcggggcggagggggctctgaggtgcagctggtggagagcggaggaggactggtgcagccaggaggctccctgcggctgtcttgcgccgccagcggctttaccatctccgactactggattcactgggtgagacaggcacctggcaagggactggagtgggtggcaggaatcaccccagcaggaggctacacatactatgccgacagcgtgaagggccggttcaccatctccgccgatacctctaagaacacagcctatctgcagatgaactccctgcgggccgaggacacagccgtgtactattgcgccagattcgtgttcttcctgccatacgccatggattattggggccagggcaccctggtgacagtgagctcc

SEQ ID NO: 47 - protein, 9 aa, synthetic construct
  REGION 1..9: note = VL VEGF-A G6-31 -CDR3
QQGYGNPFT

SEQ ID NO: 48 - protein, 108 aa, synthetic construct
  REGION 1..108: note = VL VEGF-A G6-31
DIQMTQSPSSLSASVGDRVTITCRASQDVSTAVAWYQQKPGKAPKLLIYSASFLYSGVPSRFSGSGSGTDFTLTISSLQPEDFATYYCQQGYGNPFTFGQGTKVEIKR

SEQ ID NO: 49 - protein, 496 aa, synthetic construct
  REGION 1..496: note = VH VEGF-A- (G4S)3-VL VEGF-A- G4S-VH ANG-2- (G4S)3-VL ANG-2
EVQLVESGGGLVQPGGSLRLSCAASGFTISDYWIHWVRQAPGKGLEWVAGITPAGGYTYYADSVKGRFTISADTSKNTAYLQMNSLRAEDTAVYYCARFVFFLPYAMDYWGQGTLVTVSSGGGGSGGGGSGGGGSDIQMTQSPSSLSASVGDRVTITCRASQDVSTAVAWYQQKPGKAPKLLIYSASFLYSGVPSRFSGSGSGTDFTLTISSLQPEDFATYYCQQGYGNPFTFGQGTKVEIKRGGGGSQVQLVESGGGVVQPGRSLRLSCAASGFTFTNYGMHWGRQAPGKGLEWVAVISHDGNNKYYVDSVKGRFTISRDNSKNTLYLQMNSLRAEDTAVYYCAREGIDFWSGLNWFDPWGQGTLVTVSSAGGGGSGGGGSGGGGSEIVLTQSPGTLSLSPGERATLSCRASQSITGSYLAWYQQKPGQAPRLLICGASSWATGIPDRFSGSGSGTDFTLTISRLEPEDFAVYYCQQYSSSPITFGQGTRLEIKR

SEQ ID NO: 50 - protein, 520 aa, synthetic construct
  REGION 1..520: note = CD5-sp-VH VEGF-A- (G4S)3-VL VEGF-A- G4S-VH ANG-2- (G4S)3-VL ANG-2
MPMGSLQPLATLYLLGMLVASCLGEVQLVESGGGLVQPGGSLRLSCAASGFTISDYWIHWVRQAPGKGLEWVAGITPAGGYTYYADSVKGRFTISADTSKNTAYLQMNSLRAEDTAVYYCARFVFFLPYAMDYWGQGTLVTVSSGGGGSGGGGSGGGGSDIQMTQSPSSLSASVGDRVTITCRASQDVSTAVAWYQQKPGKAPKLLIYSASFLYSGVPSRFSGSGSGTDFTLTISSLQPEDFATYYCQQGYGNPFTFGQGTKVEIKRGGGGSQVQLVESGGGVVQPGRSLRLSCAASGFTFTNYGMHWGRQAPGKGLEWVAVISHDGNNKYYVDSVKGRFTISRDNSKNTLYLQMNSLRAEDTAVYYCAREGIDFWSGLNWFDPWGQGTLVTVSSAGGGGSGGGGSGGGGSEIVLTQSPGTLSLSPGERATLSCRASQSITGSYLAWYQQKPGQAPRLLICGASSWATGIPDRFSGSGSGTDFTLTISRLEPEDFAVYYCQQYSSSPITFGQGTRLEIKR

SEQ ID NO: 51 - protein, 486 aa, synthetic construct
  REGION 1..486: note = VL ANG-2-G4S-VH VEGF-A-(G4S)3-VL VEGF-A-G4S-VH ANG-2
EIVLTQSPGTLSLSPGERATLSCRASQSITGSYLAWYQQKPGQAPRLLICGASSWATGIPDRFSGSGSGTDFTLTISRLEPEDFAVYYCQQYSSSPITFGQGTRLEIKRGGGGSEVQLVESGGGLVQPGGSLRLSCAASGFTISDYWIHWVRQAPGKGLEWVAGITPAGGYTYYADSVKGRFTISADTSKNTAYLQMNSLRAEDTAVYYCARFVFFLPYAMDYWGQGTLVTVSSGGGGSGGGGSGGGGSDIQMTQSPSSLSASVGDRVTITCRASQDVSTAVAWYQQKPGKAPKLLIYSASFLYSGVPSRFSGSGSGTDFTLTISSLQPEDFATYYCQQGYGNPFTFGQGTKVEIKRGGGGSQVQLVESGGGVVQPGRSLRLSCAASGFTFTNYGMHWGRQAPGKGLEWVAVISHDGNNKYYVDSVKGRFTISRDNSKNTLYLQMNSLRAEDTAVYYCAREGIDFWSGLNWFDPWGQGTLVTVSSA

SEQ ID NO: 52 - protein, 510 aa, synthetic construct
  REGION 1..510: note = CD5-sp-VL ANG-2-G4S-VH VEGF-A-(G4S)3-VL VEGF-A-G4S-VH ANG-2
MPMGSLQPLATLYLLGMLVASCLGEIVLTQSPGTLSLSPGERATLSCRASQSITGSYLAWYQQKPGQAPRLLICGASSWATGIPDRFSGSGSGTDFTLTISRLEPEDFAVYYCQQYSSSPITFGQGTRLEIKRGGGGSEVQLVESGGGLVQPGGSLRLSCAASGFTISDYWIHWVRQAPGKGLEWVAGITPAGGYTYYADSVKGRFTISADTSKNTAYLQMNSLRAEDTAVYYCARFVFFLPYAMDYWGQGTLVTVSSGGGGSGGGGSGGGGSDIQMTQSPSSLSASVGDRVTITCRASQDVSTAVAWYQQKPGKAPKLLIYSASFLYSGVPSRFSGSGSGTDFTLTISSLQPEDFATYYCQQGYGNPFTFGQGTKVEIKRGGGGSQVQLVESGGGVVQPGRSLRLSCAASGFTFTNYGMHWGRQAPGKGLEWVAVISHDGNNKYYVDSVKGRFTISRDNSKNTLYLQMNSLRAEDTAVYYCAREGIDFWSGLNWFDPWGQGTLVTVSSA

SEQ ID NO: 53 - protein, 486 aa, synthetic construct
  REGION 1..486: note = VL VEGF-A-G4S -VH ANG-2-(G4S)3-VL ANG-2-G4S -VH VEGF-A
DIQMTQSPSSLSASVGDRVTITCRASQDVSTAVAWYQQKPGKAPKLLIYSASFLYSGVPSRFSGSGSGTDFTLTISSLQPEDFATYYCQQGYGNPFTFGQGTKVEIKRGGGGSQVQLVESGGGVVQPGRSLRLSCAASGFTFTNYGMHWGRQAPGKGLEWVAVISHDGNNKYYVDSVKGRFTISRDNSKNTLYLQMNSLRAEDTAVYYCAREGIDFWSGLNWFDPWGQGTLVTVSSAGGGGSGGGGSGGGGSEIVLTQSPGTLSLSPGERATLSCRASQSITGSYLAWYQQKPGQAPRLLICGASSWATGIPDRFSGSGSGTDFTLTISRLEPEDFAVYYCQQYSSSPITFGQGTRLEIKRGGGGSEVQLVESGGGLVQPGGSLRLSCAASGFTISDYWIHWVRQAPGKGLEWVAGITPAGGYTYYADSVKGRFTISADTSKNTAYLQMNSLRAEDTAVYYCARFVFFLPYAMDYWGQGTLVTVSS

SEQ ID NO: 54 - protein, 510 aa, synthetic construct
  REGION 1..510: note = CD5-sp-VL VEGF-A-G4S -VH ANG-2-(G4S)3-VL ANG-2-G4S -VH VEGF-A
MPMGSLQPLATLYLLGMLVASCLGDIQMTQSPSSLSASVGDRVTITCRASQDVSTAVAWYQQKPGKAPKLLIYSASFLYSGVPSRFSGSGSGTDFTLTISSLQPEDFATYYCQQGYGNPFTFGQGTKVEIKRGGGGSQVQLVESGGGVVQPGRSLRLSCAASGFTFTNYGMHWGRQAPGKGLEWVAVISHDGNNKYYVDSVKGRFTISRDNSKNTLYLQMNSLRAEDTAVYYCAREGIDFWSGLNWFDPWGQGTLVTVSSAGGGGSGGGGSGGGGSEIVLTQSPGTLSLSPGERATLSCRASQSITGSYLAWYQQKPGQAPRLLICGASSWATGIPDRFSGSGSGTDFTLTISRLEPEDFAVYYCQQYSSSPITFGQGTRLEIKRGGGGSEVQLVESGGGLVQPGGSLRLSCAASGFTISDYWIHWVRQAPGKGLEWVAGITPAGGYTYYADSVKGRFTISADTSKNTAYLQMNSLRAEDTAVYYCARFVFFLPYAMDYWGQGTLVTVSS

SEQ ID NO: 55 - DNA, 27 bp, synthetic construct
  misc_feature 1..27: note = VL VEGF-A G6-31 -CDR3
  source 1..27: mol_type = other DNA
cagcagggctatggcaatccattcacc

SEQ ID NO: 56 - DNA, 324 bp, synthetic construct
  misc_feature 1..324: note = VL VEGF-A G6-31
  source 1..324: mol_type = other DNA
gatattcagatgacacagtccccatctagcctgtctgccagcgtgggcgacagggtgaccatcacatgtagagcaagccaggacgtgagcaccgcagtggcatggtaccagcagaagcctggcaaggccccaaagctgctgatctactccgcctctttcctgtattctggcgtgccaagcaggtttagcgggtccggatctggaaccgacttcaccctgacaatctcctctctgcagcctgaggattttgccacatactattgccagcagggctatggcaatccattcacctttggccagggcacaaaggtggagatcaagagg

SEQ ID NO: 57 - DNA, 1488 bp, synthetic construct
  misc_feature 1..1488: note = VH VEGF-A- (G4S)3-VL VEGF-A- G4S-VH ANG-2- (G4S)3-VL ANG-2
  source 1..1488: mol_type = other DNA
gaggtgcagctggtggagagcggaggaggactggtgcagccaggaggctccctgcggctgtcttgcgccgccagcggctttaccatctccgactactggattcactgggtgagacaggcacctggcaagggactggagtgggtggcaggaatcaccccagcaggaggctacacatactatgccgacagcgtgaagggccggttcaccatctccgccgatacctctaagaacacagcctatctgcagatgaactccctgcgggccgaggacacagccgtgtactattgcgccagattcgtgttcttcctgccatacgccatggattattggggccagggcaccctggtgacagtgagctccggtggaggtggctccggtggcggtggcagcggcggtggcggctctgatattcagatgacacagtccccatctagcctgtctgccagcgtgggcgacagggtgaccatcacatgtagagcaagccaggacgtgagcaccgcagtggcatggtaccagcagaagcctggcaaggccccaaagctgctgatctactccgcctctttcctgtattctggcgtgccaagcaggtttagcgggtccggatctggaaccgacttcaccctgacaatctcctctctgcagcctgaggattttgccacatactattgccagcagggctatggcaatccattcacctttggccagggcacaaaggtggagatcaagaggggcggagggggctctcaggtgcagctggttgaatctggtggcggagttgtgcagcctggcagaagcctgagactgtcttgtgccgccagcggcttcaccttcaccaactatggaatgcactggggcagacaggcccctggcaaaggacttgaatgggtcgccgtgatcagccacgacggcaacaacaagtactacgtggacagcgtgaagggcagattcaccatcagccgggacaacagcaagaacaccctgtacctgcagatgaacagcctgagagccgaggacaccgccgtgtactattgtgccagagagggcatcgacttttggagcggcctgaattggttcgacccttggggacagggcaccctggttacagtttcttctgccggtggaggtggctccggtggcggtggcagcggcggtggcggctctgagatcgtgctgacacagagccctggcacactgtcactgtctccaggcgaaagagccacactgagctgtagagccagccagagcatcaccggctcttacctggcttggtatcagcagaagcctggacaggcccctagactgctgatttgtggcgcctcttcttgggccaccggcattcccgatagattttctggcagcggctccggcaccgacttcaccctgacaatcagcagactggaacccgaggacttcgccgtgtactactgccagcagtacagcagcagccccatcacctttggccagggcacaagactggaaatcaagcgg

SEQ ID NO: 58 - DNA, 1560 bp, synthetic construct
  misc_feature 1..1560: note = CD5-sp-VH VEGF-A- (G4S)3-VL VEGF-A- G4S-VH ANG-2- (G4S)3-VL ANG-2
  source 1..1560: mol_type = other DNA
atgccaatggggtccctacaacccctggcaacactatatctgctaggtatgctcgtggcctcctgtttaggagaggtgcagctggtggagagcggaggaggactggtgcagccaggaggctccctgcggctgtcttgcgccgccagcggctttaccatctccgactactggattcactgggtgagacaggcacctggcaagggactggagtgggtggcaggaatcaccccagcaggaggctacacatactatgccgacagcgtgaagggccggttcaccatctccgccgatacctctaagaacacagcctatctgcagatgaactccctgcgggccgaggacacagccgtgtactattgcgccagattcgtgttcttcctgccatacgccatggattattggggccagggcaccctggtgacagtgagctccggtggaggtggctccggtggcggtggcagcggcggtggcggctctgatattcagatgacacagtccccatctagcctgtctgccagcgtgggcgacagggtgaccatcacatgtagagcaagccaggacgtgagcaccgcagtggcatggtaccagcagaagcctggcaaggccccaaagctgctgatctactccgcctctttcctgtattctggcgtgccaagcaggtttagcgggtccggatctggaaccgacttcaccctgacaatctcctctctgcagcctgaggattttgccacatactattgccagcagggctatggcaatccattcacctttggccagggcacaaaggtggagatcaagaggggcggagggggctctcaggtgcagctggttgaatctggtggcggagttgtgcagcctggcagaagcctgagactgtcttgtgccgccagcggcttcaccttcaccaactatggaatgcactggggcagacaggcccctggcaaaggacttgaatgggtcgccgtgatcagccacgacggcaacaacaagtactacgtggacagcgtgaagggcagattcaccatcagccgggacaacagcaagaacaccctgtacctgcagatgaacagcctgagagccgaggacaccgccgtgtactattgtgccagagagggcatcgacttttggagcggcctgaattggttcgacccttggggacagggcaccctggttacagtttcttctgccggtggaggtggctccggtggcggtggcagcggcggtggcggctctgagatcgtgctgacacagagccctggcacactgtcactgtctccaggcgaaagagccacactgagctgtagagccagccagagcatcaccggctcttacctggcttggtatcagcagaagcctggacaggcccctagactgctgatttgtggcgcctcttcttgggccaccggcattcccgatagattttctggcagcggctccggcaccgacttcaccctgacaatcagcagactggaacccgaggacttcgccgtgtactactgccagcagtacagcagcagccccatcacctttggccagggcacaagactggaaatcaagcgg

SEQ ID NO: 59 - DNA, 1458 bp, synthetic construct
  misc_feature 1..1458: note = VL ANG-2-G4S-VH VEGF-A-(G4S)3-VL VEGF-A-G4S-VH ANG-2
  source 1..1458: mol_type = other DNA
gagatcgtgctgacacagagccctggcacactgtcactgtctccaggcgaaagagccacactgagctgtagagccagccagagcatcaccggctcttacctggcttggtatcagcagaagcctggacaggcccctagactgctgatttgtggcgcctcttcttgggccaccggcattcccgatagattttctggcagcggctccggcaccgacttcaccctgacaatcagcagactggaacccgaggacttcgccgtgtactactgccagcagtacagcagcagccccatcacctttggccagggcacaagactggaaatcaagcggggcggagggggctctgaggtgcagctggtggagagcggaggaggactggtgcagccaggaggctccctgcggctgtcttgcgccgccagcggctttaccatctccgactactggattcactgggtgagacaggcacctggcaagggactggagtgggtggcaggaatcaccccagcaggaggctacacatactatgccgacagcgtgaagggccggttcaccatctccgccgatacctctaagaacacagcctatctgcagatgaactccctgcgggccgaggacacagccgtgtactattgcgccagattcgtgttcttcctgccatacgccatggattattggggccagggcaccctggtgacagtgagctccggtggaggtggctccggtggcggtggcagcggcggtggcggctctgatattcagatgacacagtccccatctagcctgtctgccagcgtgggcgacagggtgaccatcacatgtagagcaagccaggacgtgagcaccgcagtggcatggtaccagcagaagcctggcaaggccccaaagctgctgatctactccgcctctttcctgtattctggcgtgccaagcaggtttagcgggtccggatctggaaccgacttcaccctgacaatctcctctctgcagcctgaggattttgccacatactattgccagcagggctatggcaatccattcacctttggccagggcacaaaggtggagatcaagaggggcggagggggctctcaggtgcagctggttgaatctggtggcggagttgtgcagcctggcagaagcctgagactgtcttgtgccgccagcggcttcaccttcaccaactatggaatgcactggggcagacaggcccctggcaaaggacttgaatgggtcgccgtgatcagccacgacggcaacaacaagtactacgtggacagcgtgaagggcagattcaccatcagccgggacaacagcaagaacaccctgtacctgcagatgaacagcctgagagccgaggacaccgccgtgtactattgtgccagagagggcatcgacttttggagcggcctgaattggttcgacccttggggacagggcaccctggttacagtttcttctgcc

SEQ ID NO: 60 - DNA, 1530 bp, synthetic construct
  misc_feature 1..1530: note = CD5-sp-VL ANG-2-G4S-VH VEGF-A-(G4S)3-VL VEGF-A-G4S-VH ANG-2
  source 1..1530: mol_type = other DNA
atgccaatggggtccctacaacccctggcaacactatatctgctaggtatgctcgtggcctcctgtttaggagagatcgtgctgacacagagccctggcacactgtcactgtctccaggcgaaagagccacactgagctgtagagccagccagagcatcaccggctcttacctggcttggtatcagcagaagcctggacaggcccctagactgctgatttgtggcgcctcttcttgggccaccggcattcccgatagattttctggcagcggctccggcaccgacttcaccctgacaatcagcagactggaacccgaggacttcgccgtgtactactgccagcagtacagcagcagccccatcacctttggccagggcacaagactggaaatcaagcggggcggagggggctctgaggtgcagctggtggagagcggaggaggactggtgcagccaggaggctccctgcggctgtcttgcgccgccagcggctttaccatctccgactactggattcactgggtgagacaggcacctggcaagggactggagtgggtggcaggaatcaccccagcaggaggctacacatactatgccgacagcgtgaagggccggttcaccatctccgccgatacctctaagaacacagcctatctgcagatgaactccctgcgggccgaggacacagccgtgtactattgcgccagattcgtgttcttcctgccatacgccatggattattggggccagggcaccctggtgacagtgagctccggtggaggtggctccggtggcggtggcagcggcggtggcggctctgatattcagatgacacagtccccatctagcctgtctgccagcgtgggcgacagggtgaccatcacatgtagagcaagccaggacgtgagcaccgcagtggcatggtaccagcagaagcctggcaaggccccaaagctgctgatctactccgcctctttcctgtattctggcgtgccaagcaggtttagcgggtccggatctggaaccgacttcaccctgacaatctcctctctgcagcctgaggattttgccacatactattgccagcagggctatggcaatccattcacctttggccagggcacaaaggtggagatcaagaggggcggagggggctctcaggtgcagctggttgaatctggtggcggagttgtgcagcctggcagaagcctgagactgtcttgtgccgccagcggcttcaccttcaccaactatggaatgcactggggcagacaggcccctggcaaaggacttgaatgggtcgccgtgatcagccacgacggcaacaacaagtactacgtggacagcgtgaagggcagattcaccatcagccgggacaacagcaagaacaccctgtacctgcagatgaacagcctgagagccgaggacaccgccgtgtactattgtgccagagagggcatcgacttttggagcggcctgaattggttcgacccttggggacagggcaccctggttacagtttcttctgcc

SEQ ID NO: 61 - DNA, 1458 bp, synthetic construct
  misc_feature 1..1458: note = VL VEGF-A-G4S -VH ANG-2-(G4S)3-VL ANG-2-G4S -VH VEGF-A
  source 1..1458: mol_type = other DNA
gatattcagatgacacagtccccatctagcctgtctgccagcgtgggcgacagggtgaccatcacatgtagagcaagccaggacgtgagcaccgcagtggcatggtaccagcagaagcctggcaaggccccaaagctgctgatctactccgcctctttcctgtattctggcgtgccaagcaggtttagcgggtccggatctggaaccgacttcaccctgacaatctcctctctgcagcctgaggattttgccacatactattgccagcagggctatggcaatccattcacctttggccagggcacaaaggtggagatcaagaggggcggagggggctctcaggtgcagctggttgaatctggtggcggagttgtgcagcctggcagaagcctgagactgtcttgtgccgccagcggcttcaccttcaccaactatggaatgcactggggcagacaggcccctggcaaaggacttgaatgggtcgccgtgatcagccacgacggcaacaacaagtactacgtggacagcgtgaagggcagattcaccatcagccgggacaacagcaagaacaccctgtacctgcagatgaacagcctgagagccgaggacaccgccgtgtactattgtgccagagagggcatcgacttttggagcggcctgaattggttcgacccttggggacagggcaccctggttacagtttcttctgccggtggaggtggctccggtggcggtggcagcggcggtggcggctctgagatcgtgctgacacagagccctggcacactgtcactgtctccaggcgaaagagccacactgagctgtagagccagccagagcatcaccggctcttacctggcttggtatcagcagaagcctggacaggcccctagactgctgatttgtggcgcctcttcttgggccaccggcattcccgatagattttctggcagcggctccggcaccgacttcaccctgacaatcagcagactggaacccgaggacttcgccgtgtactactgccagcagtacagcagcagccccatcacctttggccagggcacaagactggaaatcaagcggggcggagggggctctgaggtgcagctggtggagagcggaggaggactggtgcagccaggaggctccctgcggctgtcttgcgccgccagcggctttaccatctccgactactggattcactgggtgagacaggcacctggcaagggactggagtgggtggcaggaatcaccccagcaggaggctacacatactatgccgacagcgtgaagggccggttcaccatctccgccgatacctctaagaacacagcctatctgcagatgaactccctgcgggccgaggacacagccgtgtactattgcgccagattcgtgttcttcctgccatacgccatggattattggggccagggcaccctggtgacagtgagctcc

SEQ ID NO: 62 - DNA, 1530 bp, synthetic construct
  misc_feature 1..1530: note = CD5-sp-VL VEGF-A-G4S -VH ANG-2-(G4S)3-VL ANG-2-G4S -VH VEGF-A
  source 1..1530: mol_type = other DNA
atgccaatggggtccctacaacccctggcaacactatatctgctaggtatgctcgtggcctcctgtttaggagatattcagatgacacagtccccatctagcctgtctgccagcgtgggcgacagggtgaccatcacatgtagagcaagccaggacgtgagcaccgcagtggcatggtaccagcagaagcctggcaaggccccaaagctgctgatctactccgcctctttcctgtattctggcgtgccaagcaggtttagcgggtccggatctggaaccgacttcaccctgacaatctcctctctgcagcctgaggattttgccacatactattgccagcagggctatggcaatccattcacctttggccagggcacaaaggtggagatcaagaggggcggagggggctctcaggtgcagctggttgaatctggtggcggagttgtgcagcctggcagaagcctgagactgtcttgtgccgccagcggcttcaccttcaccaactatggaatgcactggggcagacaggcccctggcaaaggacttgaatgggtcgccgtgatcagccacgacggcaacaacaagtactacgtggacagcgtgaagggcagattcaccatcagccgggacaacagcaagaacaccctgtacctgcagatgaacagcctgagagccgaggacaccgccgtgtactattgtgccagagagggcatcgacttttggagcggcctgaattggttcgacccttggggacagggcaccctggttacagtttcttctgccggtggaggtggctccggtggcggtggcagcggcggtggcggctctgagatcgtgctgacacagagccctggcacactgtcactgtctccaggcgaaagagccacactgagctgtagagccagccagagcatcaccggctcttacctggcttggtatcagcagaagcctggacaggcccctagactgctgatttgtggcgcctcttcttgggccaccggcattcccgatagattttctggcagcggctccggcaccgacttcaccctgacaatcagcagactggaacccgaggacttcgccgtgtactactgccagcagtacagcagcagccccatcacctttggccagggcacaagactggaaatcaagcggggcggagggggctctgaggtgcagctggtggagagcggaggaggactggtgcagccaggaggctccctgcggctgtcttgcgccgccagcggctttaccatctccgactactggattcactgggtgagacaggcacctggcaagggactggagtgggtggcaggaatcaccccagcaggaggctacacatactatgccgacagcgtgaagggccggttcaccatctccgccgatacctctaagaacacagcctatctgcagatgaactccctgcgggccgaggacacagccgtgtactattgcgccagattcgtgttcttcctgccatacgccatggattattggggccagggcaccctggtgacagtgagctcc